European Patent Specification EP 3 735 471 B1, published June 28, 2023. Title: METHOD. Applicant: OXFORD NANOPORE TECHNOLOGIES LIMITED. The sequence listing filed with the application follows.

SEQUENCE LISTING (6 sequences)

SEQ ID NO: 1 - DNA, 63 bp, Artificial Sequence
  Size Selection Adapter Top Strand
  misc_feature (1)..(1): 5Phos
ggcgtctgcttgggtgtttaaccttttttttttttaatgtacttcgttcagttacgtattgct

SEQ ID NO: 2 - DNA, 29 bp, Artificial Sequence
  Size Selection Adapter Bottom Strand
  misc_feature (1)..(1): 5Phos
gcaatacgtaactgaacgaagtacatttt

SEQ ID NO: 3 - DNA, 29 bp, Artificial Sequence
  Blocker Strand Example 1
ggttaaacacccaagcagacgccagcaat

SEQ ID NO: 4 - protein, 148 aa, Artificial Sequence
  strep-SUMO tag
MGGSAWSHPQFEKGGGSGGGSGGSAWSHPQFEKSGGGGGSDSEVNQEAKPEVKPEVKPETHINLKVSDGSSEIFFKIKKTTPLRRLMEAFAKRQGKEMDSLRFLYDGIRIQADQTPEDLDMEDNDIIEAHREQIGGSTSGSGENLYFQ

SEQ ID NO: 5 - DNA, 3561 bp, Artificial Sequence
  3.6kb DNA
gccatcagattgtgtttgttagtcgctttttttttttggaattttttttttggaattttttttttgcgctaacaacctcctgccgttttgcccgtgcatatcggtcacgaacaaatctgattactaaacacagtagcctggatttgttctatcagtaatcgaccttattcctaattaaatagagcaaatccccttattgggggtaagacatgaagatgccagaaaaacatgacctgttggccgccattctcgcggcaaaggaacaaggcatcggggcaatccttgcgtttgcaatggcgtaccttcgcggcagatataatggcggtgcgtttacaaaaacagtaatcgacgcaacgatgtgcgccattatcgcctagttcattcgtgaccttctcgacttcgccggactaagtagcaatctcgcttatataacgagcgtgtttatcggctacatcggtactgactcgattggttcgcttatcaaacgcttcgctgctaaaaaagccggagtagaagatggtagaaatcaataatcaacgtaaggcgttcctcgatatgctggcgtggtcggagggaactgataacggacgtcagaaaaccagaaatcatggttatgacgtcattgtaggcggagagctatttactgattactccgatcaccctcgcaaacttgtcacgctaaacccaaaactcaaatcaacaggcgccggacgctaccagcttctttcccgttggtgggatgcctaccgcaagcagcttggcctgaaagacttctctccgaaaagtcaggacgctgtggcattgcagcagattaaggagcgtggcgctttacctatgattgatcgtggtgatatccgtcaggcaatcgaccgttgcagcaatatctgggcttcactgccgggcgctggttatggtcagttcgagcataaggctgacagcctgattgcaaaattcaaagaagcgggcggaacggtcagagagattgatgtatgagcagagtcaccgcgattatctccgctctggttatctgcatcatcgtctgcctgtcatgggctgttaatcattaccgtgataacgccattacctacaaagcccagcgcgacaaaaatgccagagaactgaagctggcgaacgcggcaattactgacatgcagatgcgtcagcgtgatgttgctgcgctcgatgcaaaatacacgaaggagttagctgatgctaaagctgaaaatgatgctctgcgtgatgatgttgccgctggtcgtcgtcggttgcacatcaaagcagtctgtcagtcagtgcgtgaagccaccaccgcctccggcgtggataatgcagcctccccccgactggcagacaccgctgaacgggattatttcaccctcagagagaggctgatcactatgcaaaaacaactggaaggaacccagaagtatattaatgagcagtgcagatagagttgcccatatcgatgggcaactcatgcaattattgtgagcaatacacacgcgcttccagcggagtataaatgcctaaagtaataaaaccgagcaatccatttacgaatgtttgctgggtttctgttttaacaacattttctgcgccgccacaaattttggctgcatcgacagttttcttctgcccaattccagaaacgaagaaatgatgggtgatggtttcctttggtgctactgctgccggtttgttttgaacagtaaacgtctgttgagcacatcctgtaataagcagggccagcgcagtagcgagtagcatttttttcatggtgttattcccgatgctttttgaagttcgcagaatcgtatgtgtagaaaattaaacaaaccctaaacaatgagttgaaatttcatattgttaatatttattaatgtatgtcaggtgcgatgaatcgtcattgtattcccggattaactatgtccacagccctgacggggaacttctctgcgggagtgtccgggaataattaaaacgatgcacacagggtttagcgcgtacacgtattgcattatgccaacgccccggtgctgacacggaagaaaccggacgttatgatttagcgtggaaagatttgtgtagtgttctgaatgctctcagtaaatagtaatgaattatcaaaggtatagtaatatcttttatgttcatggatatttgtaacccatcggaaaactcctgctttagcaagattttccctgtattgctgaaatgtgatttctcttgatttcaacctatcataggacgtttctataagatgcgtgtttcttgagaatttaacatttacaacctttttaagtccttttattaacacggtgttatcgttttctaacacgatgtgaatattatctgtggctagatagtaaatataatgtgagacgttgtgacgttttagttcagaataaaacaattcacagtctaaatcttttcgcacttgatcgaatatttctttaaaaatggcaacctgagccattggtaaaaccttccatgtgatacgagggcgcgtagtttgcattatcgtttttatcgtttcaatctggtctgacctccttgtgttttgttgatgatttatgtcaaatattaggaatgttttcacttaatagtattggttgcgtaacaaagtgcggtcctgctggcattctggagggaaatacaaccgacagatgtatgtaaggccaacgtgctcaaatcttcatacagaaagatttgaagtaatattttaaccgctagatgaagagcaagcgcatggagcgacaaaatgaataaagaacaatctgctgatgatccctccgtggatctgattcgtgtaaaaaatatgcttaatagcaccatttctatgagttaccctgatgttgtaattgcatgtatagaacataaggtgtctctggaagcattcagagcaattgaggcagcgttggtgaagcacgataataatatgaaggattattccctggtggttgactgatcaccataactgctaatcattcaaactatttagtctgtgacagagccaacacgcagtctgtcactgtcaggaaagtggtaaaactgcaactcaattactgcaatgccctcgtaattaagtgaatttacaatatcgtcctgttcggagggaagaacgcgggatgttcattcttcatcacttttaattgatgtatatgctctcttttctgacgttagtctccgacggcaggcttcaatgacccaggctgagaaattcccggaccctttttgctcaagagcgatgttaatttgttcaatcatttggttaggaaagcggatgttgcgggttgttgttctgcgggttctgttcttcgttgacatgaggttgccccgtattcagtgtcgctgatttgtattgtctgaagttgtttttacgttaagttgatgcagatcaattaatacgatacctgcgtcataattgattatttgacgtggtttgatggcctccacgcacgttgtgatatgtagatgataatcattatcactttacgggtcctttccggtgaaaaaaaaggtaccaaaaaaaacatcgtcgtgagtagtgaaccgtaagca

SEQ ID NO: 6 - DNA, 28 bp, Artificial Sequence
  Blocker Strand Example 2
  misc_feature (1)..(1): 5'BNA-G
  misc_feature (2)..(2): iBNA-G
  misc_feature (3)..(4): iBNA-T
  misc_feature (5)..(5): iBNA-A
ggttaaacacccaagcagacgccagcaa